European Patent Application EP 4 585 272 A2, published July 16, 2025. Title: LIPID NANOPARTICLE FORMULATIONS FOR CRISPR/CAS COMPONENTS. Applicant: Intellia Therapeutics, Inc. The sequence listing filed with the application follows.

SEQUENCE LISTING (164 sequences)

SEQ ID NO: 1 - protein, 7 aa, Simian virus 40
PKKKRKV

SEQ ID NO: 2 - protein, 7 aa, Simian virus 40
PKKKRRV

SEQ ID NO: 3 - protein, 16 aa, unidentified
  REGION 1..16: note = source = /note="Description of Unknown: Nucleoplasmin bipartite NLS sequence"
KRPAATKKAGQAKKKK

SEQ ID NO: 4 - protein, 6 aa, synthetic construct
  REGION 1..6: note = source = /note="Description of Artificial Sequence: Synthetic 6xHis tag"
HHHHHH

SEQ ID NO: 5 - protein, 8 aa, synthetic construct
  REGION 1..8: note = source = /note="Description of Artificial Sequence: Synthetic 8xHis tag"
HHHHHHHH

SEQ ID NO: 6 - RNA, 100 nt, synthetic construct
  misc_feature 1..100: note = source = /note="Description of Artificial Sequence: Synthetic polynucleotide"
  source 1..100: mol_type = other RNA
ttacagccacgtctacagcagttttagagctagaaatagcaagttaaaataaggctagtccgttatcaacttgaaaaagtggcaccgagtcggtgctttt

SEQ ID NO: 7 - RNA, 100 nt, synthetic construct
  misc_feature 1..100: note = source = /note="Description of Artificial Sequence: Synthetic polynucleotide"
  source 1..100: mol_type = other RNA
gctgccaggaacctacattggttttagagctagaaatagcaagttaaaataaggctagtccgttatcaacttgaaaaagtggcaccgagtcggtgctttt

SEQ ID NO: 8 - RNA, 4603 nt, synthetic construct
  misc_feature 1..4603: note = source = /note="Description of Artificial Sequence: Synthetic polynucleotide"
  source 1..4603: mol_type = other RNA
gggtcccgcagtcggcgtccagcggctctgcttgttcgtgtgtgtgtcgttgcaggccttattcggatccatggataagaagtactcaatcgggctggatatcggaactaattccgtgggttgggcagtgatcacggatgaatacaaagtgccgtccaagaagttcaaggtcctggggaacaccgatagacacagcatcaagaaaaatctcatcggagccctgctgtttgactccggcgaaaccgcagaagcgacccggctcaaacgtaccgcgaggcgacgctacacccggcggaagaatcgcatctgctatctgcaagagatcttttcgaacgaaatggcaaaggtcgacgacagcttcttccaccgcctggaagaatctttcctggtggaggaggacaagaagcatgaacggcatcctatctttggaaacatcgtcgacgaagtggcgtaccacgaaaagtacccgaccatctaccatctgcggaagaagttggttgactcaactgacaaggccgacctcagattgatctacttggccctcgcccatatgatcaaattccgcggacacttcctgatcgaaggcgatctgaaccctgataactccgacgtggataagcttttcattcaactggtgcagacctacaaccaactgttcgaagaaaacccaatcaatgctagcggcgtcgatgccaaggccatcctgtccgcccggctgtcgaagtcgcggcgcctcgaaaacctgatcgcacagctgccgggagagaaaaagaacggacttttcggcaacttgatcgctctctcactgggactcactcccaatttcaagtccaattttgacctggccgaggacgcgaagctgcaactctcaaaggacacctacgacgacgacttggacaatttgctggcacaaattggcgatcagtacgcggatctgttccttgccgctaagaacctttcggacgcaatcttgctgtccgatatcctgcgcgtgaacaccgaaataaccaaagcgccgcttagcgcctcgatgattaagcggtacgacgagcatcaccaggatctcacgctgctcaaagcgctcgtgagacagcaactgcctgaaaagtacaaggagatcttcttcgaccagtccaagaatgggtacgcagggtacatcgatggaggcgctagccaggaagagttctataagttcatcaagccaatcctggaaaagatggacggaaccgaagaactgctggtcaagctgaacagggaggatctgctccggaaacagagaacctttgacaacggatccattccccaccagatccatctgggtgagctgcacgccatcttgcggcgccaggaggacttttacccattcctcaaggacaaccgggaaaagatcgagaaaattctgacgttccgcatcccgtattacgtgggcccactggcgcgcggcaattcgcgcttcgcgtggatgactagaaaatcagaggaaaccatcactccttggaatttcgaggaagttgtggataagggagcttcggcacaaagcttcatcgaacgaatgaccaacttcgacaagaatctcccaaacgagaaggtgcttcctaagcacagcctcctttacgaatacttcactgtctacaacgaactgactaaagtgaaatacgttactgaaggaatgaggaagccggcctttctgtccggagaacagaagaaagcaattgtcgatctgctgttcaagaccaaccgcaaggtgaccgtcaagcagcttaaagaggactacttcaagaagatcgagtgtttcgactcagtggaaatcagcggggtggaggacagattcaacgcttcgctgggaacctatcatgatctcctgaagatcatcaaggacaaggacttccttgacaacgaggagaacgaggacatcctggaagatatcgtcctgaccttgacccttttcgaggatcgcgagatgatcgaggagaggcttaagacctacgctcatctcttcgacgataaggtcatgaaacaactcaagcgccgccggtacactggttggggccgcctctcccgcaagctgatcaacggtattcgcgataaacagagcggtaaaactatcctggatttcctcaaatcggatggcttcgctaatcgtaacttcatgcaattgatccacgacgacagcctgacctttaaggaggacatccaaaaagcacaagtgtccggacagggagactcactccatgaacacatcgcgaatctggccggttcgccggcgattaagaagggaattctgcaaactgtgaaggtggtcgacgagctggtgaaggtcatgggacggcacaaaccggagaatatcgtgattgaaatggcccgagaaaaccagactacccagaagggccagaaaaactcccgcgaaaggatgaagcggatcgaagaaggaatcaaggagctgggcagccagatcctgaaagagcacccggtggaaaacacgcagctgcagaacgagaagctctacctgtactatttgcaaaatggacgggacatgtacgtggaccaagagctggacatcaatcggttgtctgattacgacgtggaccacatcgttccacagtcctttctgaaggatgactcgatcgataacaaggtgttgactcgcagcgacaagaacagagggaagtcagataatgtgccatcggaggaggtcgtgaagaagatgaagaattactggcggcagctcctgaatgcgaagctgattacccagagaaagtttgacaatctcactaaagccgagcgcggcggactctcagagctggataaggctggattcatcaaacggcagctggtcgagactcggcagattaccaagcacgtggcgcagatcttggactcccgcatgaacactaaatacgacgagaacgataagctcatccgggaagtgaaggtgattaccctgaaaagcaaacttgtgtcggactttcggaaggactttcagttttacaaagtgagagaaatcaacaactaccatcacgcgcatgacgcatacctcaacgctgtggtcggtaccgccctgatcaaaaagtaccctaaacttgaatcggagtttgtgtacggagactacaaggtctacgacgtgaggaagatgatagccaagtccgaacaggaaatcgggaaagcaactgcgaaatacttcttttactcaaacatcatgaactttttcaagactgaaattacgctggccaatggagaaatcaggaagaggccactgatcgaaactaacggagaaacgggcgaaatcgtgtgggacaagggcagggacttcgcaactgttcgcaaagtgctctctatgccgcaagtcaatattgtgaagaaaaccgaagtgcaaaccggcggattttcaaaggaatcgatcctcccaaagagaaatagcgacaagctcattgcacgcaagaaagactgggacccgaagaagtacggaggattcgattcgccgactgtcgcatactccgtcctcgtggtggccaaggtggagaagggaaagagcaaaaagctcaaatccgtcaaagagctgctggggattaccatcatggaacgatcctcgttcgagaagaacccgattgatttcctcgaggcgaagggttacaaggaggtgaagaaggatctgatcatcaaactccccaagtactcactgttcgaactggaaaatggtcggaagcgcatgctggcttcggccggagaactccaaaaaggaaatgagctggccttgcctagcaagtacgtcaacttcctctatcttgcttcgcactacgaaaaactcaaagggtcaccggaagataacgaacagaagcagcttttcgtggagcagcacaagcattatctggatgaaatcatcgaacaaatctccgagttttcaaagcgcgtgatcctcgccgacgccaacctcgacaaagtcctgtcggcctacaataagcatagagataagccgatcagagaacaggccgagaacattatccacttgttcaccctgactaacctgggagccccagccgccttcaagtacttcgatactactatcgatcgcaaaagatacacgtccaccaaggaagttctggacgcgaccctgatccaccaaagcatcactggactctacgaaactaggatcgatctgtcgcagctgggtggcgatggctcggcttacccatacgacgtgcctgactacgcctcgctcggatcgggctcccccaaaaagaaacggaaggtggacggatccccgaaaaagaagagaaaggtggactccggatgagaattatgcagtctagccatcacatttaaaagcatctcagcctaccatgagaataagagaaagaaaatgaagatcaatagcttattcatctctttttctttttcgttggtgtaaagccaacaccctgtctaaaaaacataaatttctttaatcattttgcctcttttctctgtgcttcaattaataaaaaatggaaagaacctcgagaaaaaaaaaaaaaaaaaaaaaaaaaaaaaaaaaaaaaaaaaaaaaaaaaaaaaaaaaaaaaaaaaaaaaaaaaaaaaaaaaaaaaaaaaaaaaaaaaaaatctag

SEQ ID NO: 9 - RNA, 4514 nt, synthetic construct
  misc_feature 1..4514: note = source = /note="Description of Artificial Sequence: Synthetic polynucleotide"
  source 1..4514: mol_type = other RNA
gggtcccgcagtcggcgtccagcggctctgcttgttcgtgtgtgtgtcgttgcaggccttattcggatccatggataagaagtactcaatcgggctggatatcggaactaattccgtgggttgggcagtgatcacggatgaatacaaagtgccgtccaagaagttcaaggtcctggggaacaccgatagacacagcatcaagaaaaatctcatcggagccctgctgtttgactccggcgaaaccgcagaagcgacccggctcaaacgtaccgcgaggcgacgctacacccggcggaagaatcgcatctgctatctgcaagagatcttttcgaacgaaatggcaaaggtcgacgacagcttcttccaccgcctggaagaatctttcctggtggaggaggacaagaagcatgaacggcatcctatctttggaaacatcgtcgacgaagtggcgtaccacgaaaagtacccgaccatctaccatctgcggaagaagttggttgactcaactgacaaggccgacctcagattgatctacttggccctcgcccatatgatcaaattccgcggacacttcctgatcgaaggcgatctgaaccctgataactccgacgtggataagcttttcattcaactggtgcagacctacaaccaactgttcgaagaaaacccaatcaatgctagcggcgtcgatgccaaggccatcctgtccgcccggctgtcgaagtcgcggcgcctcgaaaacctgatcgcacagctgccgggagagaaaaagaacggacttttcggcaacttgatcgctctctcactgggactcactcccaatttcaagtccaattttgacctggccgaggacgcgaagctgcaactctcaaaggacacctacgacgacgacttggacaatttgctggcacaaattggcgatcagtacgcggatctgttccttgccgctaagaacctttcggacgcaatcttgctgtccgatatcctgcgcgtgaacaccgaaataaccaaagcgccgcttagcgcctcgatgattaagcggtacgacgagcatcaccaggatctcacgctgctcaaagcgctcgtgagacagcaactgcctgaaaagtacaaggagatcttcttcgaccagtccaagaatgggtacgcagggtacatcgatggaggcgctagccaggaagagttctataagttcatcaagccaatcctggaaaagatggacggaaccgaagaactgctggtcaagctgaacagggaggatctgctccggaaacagagaacctttgacaacggatccattccccaccagatccatctgggtgagctgcacgccatcttgcggcgccaggaggacttttacccattcctcaaggacaaccgggaaaagatcgagaaaattctgacgttccgcatcccgtattacgtgggcccactggcgcgcggcaattcgcgcttcgcgtggatgactagaaaatcagaggaaaccatcactccttggaatttcgaggaagttgtggataagggagcttcggcacaaagcttcatcgaacgaatgaccaacttcgacaagaatctcccaaacgagaaggtgcttcctaagcacagcctcctttacgaatacttcactgtctacaacgaactgactaaagtgaaatacgttactgaaggaatgaggaagccggcctttctgtccggagaacagaagaaagcaattgtcgatctgctgttcaagaccaaccgcaaggtgaccgtcaagcagcttaaagaggactacttcaagaagatcgagtgtttcgactcagtggaaatcagcggggtggaggacagattcaacgcttcgctgggaacctatcatgatctcctgaagatcatcaaggacaaggacttccttgacaacgaggagaacgaggacatcctggaagatatcgtcctgaccttgacccttttcgaggatcgcgagatgatcgaggagaggcttaagacctacgctcatctcttcgacgataaggtcatgaaacaactcaagcgccgccggtacactggttggggccgcctctcccgcaagctgatcaacggtattcgcgataaacagagcggtaaaactatcctggatttcctcaaatcggatggcttcgctaatcgtaacttcatgcaattgatccacgacgacagcctgacctttaaggaggacatccaaaaagcacaagtgtccggacagggagactcactccatgaacacatcgcgaatctggccggttcgccggcgattaagaagggaattctgcaaactgtgaaggtggtcgacgagctggtgaaggtcatgggacggcacaaaccggagaatatcgtgattgaaatggcccgagaaaaccagactacccagaagggccagaaaaactcccgcgaaaggatgaagcggatcgaagaaggaatcaaggagctgggcagccagatcctgaaagagcacccggtggaaaacacgcagctgcagaacgagaagctctacctgtactatttgcaaaatggacgggacatgtacgtggaccaagagctggacatcaatcggttgtctgattacgacgtggaccacatcgttccacagtcctttctgaaggatgactcgatcgataacaaggtgttgactcgcagcgacaagaacagagggaagtcagataatgtgccatcggaggaggtcgtgaagaagatgaagaattactggcggcagctcctgaatgcgaagctgattacccagagaaagtttgacaatctcactaaagccgagcgcggcggactctcagagctggataaggctggattcatcaaacggcagctggtcgagactcggcagattaccaagcacgtggcgcagatcttggactcccgcatgaacactaaatacgacgagaacgataagctcatccgggaagtgaaggtgattaccctgaaaagcaaacttgtgtcggactttcggaaggactttcagttttacaaagtgagagaaatcaacaactaccatcacgcgcatgacgcatacctcaacgctgtggtcggtaccgccctgatcaaaaagtaccctaaacttgaatcggagtttgtgtacggagactacaaggtctacgacgtgaggaagatgatagccaagtccgaacaggaaatcgggaaagcaactgcgaaatacttcttttactcaaacatcatgaactttttcaagactgaaattacgctggccaatggagaaatcaggaagaggccactgatcgaaactaacggagaaacgggcgaaatcgtgtgggacaagggcagggacttcgcaactgttcgcaaagtgctctctatgccgcaagtcaatattgtgaagaaaaccgaagtgcaaaccggcggattttcaaaggaatcgatcctcccaaagagaaatagcgacaagctcattgcacgcaagaaagactgggacccgaagaagtacggaggattcgattcgccgactgtcgcatactccgtcctcgtggtggccaaggtggagaagggaaagagcaaaaagctcaaatccgtcaaagagctgctggggattaccatcatggaacgatcctcgttcgagaagaacccgattgatttcctcgaggcgaagggttacaaggaggtgaagaaggatctgatcatcaaactccccaagtactcactgttcgaactggaaaatggtcggaagcgcatgctggcttcggccggagaactccaaaaaggaaatgagctggccttgcctagcaagtacgtcaacttcctctatcttgcttcgcactacgaaaaactcaaagggtcaccggaagataacgaacagaagcagcttttcgtggagcagcacaagcattatctggatgaaatcatcgaacaaatctccgagttttcaaagcgcgtgatcctcgccgacgccaacctcgacaaagtcctgtcggcctacaataagcatagagataagccgatcagagaacaggccgagaacattatccacttgttcaccctgactaacctgggagccccagccgccttcaagtacttcgatactactatcgatcgcaaaagatacacgtccaccaaggaagttctggacgcgaccctgatccaccaaagcatcactggactctacgaaactaggatcgatctgtcgcagctgggtggcgatggcggtggatctccgaaaaagaagagaaaggtgtaatgagctagccatcacatttaaaagcatctcagcctaccatgagaataagagaaagaaaatgaagatcaatagcttattcatctctttttctttttcgttggtgtaaagccaacaccctgtctaaaaaacataaatttctttaatcattttgcctcttttctctgtgcttcaattaataaaaaatggaaagaacctcgagaaaaaaaaaaaaaaaaaaaaaaaaaaaaaaaaaaaaaaaaaaaaaaaaaaaaaaaaaaaaaaaaaaaaaaaaaaaaaaaaaaaaaaaaaaaaaaaaaaaatctag

SEQ ID NO: 10 - RNA, 74 nt, synthetic construct
  misc_feature 1..74: note = source = /note="Description of Artificial Sequence: Synthetic oligonucleotide"
  source 1..74: mol_type = other RNA
aacagcatagcaagttaaaataaggctagtccgttatcaacttgaaaaagtggcaccgagtcggtgcttttttt

SEQ ID NO: 11 - RNA, 42 nt, synthetic construct
  misc_feature 1..42: note = source = /note="Description of Artificial Sequence: Synthetic oligonucleotide"
  source 1..42: mol_type = other RNA
agggctcttgaagatctcccgttttagagctatgctgttttg

SEQ ID NO: 12 - RNA, 103 nt, synthetic construct
  misc_feature 1..103: note = source = /note="Description of Artificial Sequence: Synthetic polynucleotide"
  source 1..103: mol_type = other RNA
agggctcttgaagatctcccgttttagagctagaaatagcaagttaaaataaggctagtccgttatcaacttgaaaaagtggcaccgagtcggtgcttttttt

SEQ ID NO: 13 - RNA, 42 nt, synthetic construct
  misc_feature 1..42: note = source = /note="Description of Artificial Sequence: Synthetic oligonucleotide"
  source 1..42: mol_type = other RNA
ccagtccagcgaggcaaagggttttagagctatgctgttttg

SEQ ID NO: 14 - RNA, 105 nt, synthetic construct
  misc_feature 1..105: note = source = /note="Description of Artificial Sequence: Synthetic polynucleotide"
  source 1..105: mol_type = other RNA
ggccagtccagcgaggcaaagggttttagagctagaaatagcaagttaaaataaggctagtccgttatcaacttgaaaaagtggcaccgagtcggtgcttttttt

SEQ ID NO: 15 - RNA, 100 nt, synthetic construct
  misc_feature 1..100: note = source = /note="Description of Artificial Sequence: Synthetic polynucleotide"
  source 1..100: mol_type = other RNA
ccagtccagcgaggcaaagggttttagagctagaaatagcaagttaaaataaggctagtccgttatcaacttgaaaaagtggcaccgagtcggtgctttt

SEQ ID NO: 16 - RNA, 100 nt, synthetic construct
  misc_feature 1..100: note = source = /note="Description of Artificial Sequence: Synthetic polynucleotide"
  source 1..100: mol_type = other RNA
ctcagttttcataacccagggttttagagctagaaatagcaagttaaaataaggctagtccgttatcaacttgaaaaagtggcaccgagtcggtgctttt

SEQ ID NO: 17 - RNA, 100 nt, synthetic construct
  misc_feature 1..100: note = source = /note="Description of Artificial Sequence: Synthetic polynucleotide"
  source 1..100: mol_type = other RNA
cagggctcttgaagatctccgttttagagctagaaatagcaagttaaaataaggctagtccgttatcaacttgaaaaagtggcaccgagtcggtgctttt

SEQ ID NO: 18 - RNA, 100 nt, synthetic construct
  misc_feature 1..100: note = source = /note="Description of Artificial Sequence: Synthetic polynucleotide"
  source 1..100: mol_type = other RNA
ctttctacaagcttacccaggttttagagctagaaatagcaagttaaaataaggctagtccgttatcaacttgaaaaagtggcaccgagtcggtgctttt

SEQ ID NO: 19 - RNA, 100 nt, synthetic construct; identical to SEQ ID NO: 6
  misc_feature 1..100: note = source = /note="Description of Artificial Sequence: Synthetic polynucleotide"
  source 1..100: mol_type = other RNA

SEQ ID NO: 20 - RNA, 74 nt, synthetic construct; identical to SEQ ID NO: 10
  misc_feature 1..74: note = source = /note="Description of Artificial Sequence: Synthetic oligonucleotide"
  source 1..74: mol_type = other RNA

SEQ ID NO: 21 - RNA, 42 nt, synthetic construct; identical to SEQ ID NO: 11
  misc_feature 1..42: note = source = /note="Description of Artificial Sequence: Synthetic oligonucleotide"
  source 1..42: mol_type = other RNA

SEQ ID NO: 22 - RNA, 42 nt, synthetic construct; identical to SEQ ID NO: 13
  misc_feature 1..42: note = source = /note="Description of Artificial Sequence: Synthetic oligonucleotide"
  source 1..42: mol_type = other RNA

SEQ ID NO: 23 - RNA, 100 nt, synthetic construct
  misc_feature 1..100: note = source = /note="Description of Artificial Sequence: Synthetic polynucleotide"
  source 1..100: mol_type = other RNA
agggctcttgaagatctcccgttttagagctagaaatagcaagttaaaataaggctagtccgttatcaacttgaaaaagtggcaccgagtcggtgctttt

SEQ ID NO: 24 - RNA, 100 nt, synthetic construct; identical to SEQ ID NO: 15
  misc_feature 1..100: note = source = /note="Description of Artificial Sequence: Synthetic polynucleotide"
  source 1..100: mol_type = other RNA

SEQ ID NO: 25 - RNA, 100 nt, synthetic construct; identical to SEQ ID NO: 16
  misc_feature 1..100: note = source = /note="Description of Artificial Sequence: Synthetic polynucleotide"
  source 1..100: mol_type = other RNA

SEQ ID NO: 26 - RNA, 100 nt, synthetic construct; identical to SEQ ID NO: 17
  misc_feature 1..100: note = source = /note="Description of Artificial Sequence: Synthetic polynucleotide"
  source 1..100: mol_type = other RNA

SEQ ID NO: 27 - RNA, 100 nt, synthetic construct; identical to SEQ ID NO: 18
  misc_feature 1..100: note = source = /note="Description of Artificial Sequence: Synthetic polynucleotide"
  source 1..100: mol_type = other RNA

SEQ ID NO: 28 - RNA, 100 nt, synthetic construct; identical to SEQ ID NO: 6
  misc_feature 1..100: note = source = /note="Description of Artificial Sequence: Synthetic polynucleotide"
  source 1..100: mol_type = other RNA

SEQ ID NO: 29 - DNA, 591 bp, synthetic construct
  misc_feature 1..591: note = source = /note="Description of Artificial Sequence: Synthetic polynucleotide"
  source 1..591: mol_type = other DNA
gctgcaaggcgattaagttgggtaacgccagggttttcccagtcacgacgttgtaaaacgacggccagtgaattcgagggcctattttcccatgattccttcatatttgcatatacgatacaaggctgttagagagataattggaattaatttgactgtaaacacaaagatattagtacaaaatacgtgacgtagaaagtaataatttcttgggtagtttgcagttttaaaattatgttttaaaatggactatcatatgcttaccgtaacttgaaagtatttcgatttcttggctttatatatcttgtggaaaggacgaaacaccgctttctacaagcttacccaggttttagagctagaaatagcaagttaaaataaggctagtccgttatcaacttgaaaaagtggcaccgagtcggtgctttttttggtacccggggatcctctagagtcgacctgcaggcatgcaagcttggcgtaatcatggtcatagctgtttcctgtgtgaaattgttatccgctcacaattccacacaacatacgagccggaagcataaagtgtaaagcctggggtgcctaatgagtgagcta

SEQ ID NO: 30 - DNA, 56 bp, synthetic construct
  misc_feature 1..56: note = source = /note="Description of Artificial Sequence: Synthetic primer"
  source 1..56: mol_type = other DNA
cactctttccctacacgacgctcttccgatctgatccagtgtggctgtttccattc

SEQ ID NO: 31 - DNA, 52 bp, synthetic construct
  misc_feature 1..52: note = source = /note="Description of Artificial Sequence: Synthetic primer"
  source 1..52: mol_type = other DNA
ggagttcagacgtgtgctcttccgatctttacacaagagcaggcacgagatg

SEQ ID NO: 32 - DNA, 56 bp, synthetic construct
  misc_feature 1..56: note = source = /note="Description of Artificial Sequence: Synthetic primer"
  source 1..56: mol_type = other DNA
cactctttccctacacgacgctcttccgatctagcacatgagaccttctgtttctc

SEQ ID NO: 33 - DNA, 52 bp, synthetic construct
  misc_feature 1..52: note = source = /note="Description of Artificial Sequence: Synthetic primer"
  source 1..52: mol_type = other DNA
ggagttcagacgtgtgctcttccgatctgacataggtgtgaccctcacaatc

SEQ ID NO: 34 - DNA, 56 bp, synthetic construct; identical to SEQ ID NO: 32
  misc_feature 1..56: note = source = /note="Description of Artificial Sequence: Synthetic primer"
  source 1..56: mol_type = other DNA

SEQ ID NO: 35 - DNA, 52 bp, synthetic construct; identical to SEQ ID NO: 33
  misc_feature 1..52: note = source = /note="Description of Artificial Sequence: Synthetic primer"
  source 1..52: mol_type = other DNA

SEQ ID NO: 36 - DNA, 56 bp, synthetic construct
  misc_feature 1..56: note = source = /note="Description of Artificial Sequence: Synthetic primer"
  source 1..56: mol_type = other DNA
cactctttccctacacgacgctcttccgatctagtcaataatcagaatcagcaggt

SEQ ID NO: 37 - DNA, 55 bp, synthetic construct
  misc_feature 1..55: note = source = /note="Description of Artificial Sequence: Synthetic primer"
  source 1..55: mol_type = other DNA
ggagttcagacgtgtgctcttccgatctagaaggcacttcttctttatctaaggt

SEQ ID NO: 38 - DNA, 55 bp, synthetic construct
  misc_feature 1..55: note = source = /note="Description of Artificial Sequence: Synthetic primer"
  source 1..55: mol_type = other DNA
cactctttccctacacgacgctcttccgatcttgctggagaatccaaatgtcctc

SEQ ID NO: 39 - DNA, 55 bp, synthetic construct
  misc_feature 1..55: note = source = /note="Description of Artificial Sequence: Synthetic primer"
  source 1..55: mol_type = other DNA
ggagttcagacgtgtgctcttccgatctgctaggaattaaacctgtgtctcttac

SEQ ID NO: 40 - DNA, 56 bp, synthetic construct
  misc_feature 1..56: note = source = /note="Description of Artificial Sequence: Synthetic primer"
  source 1..56: mol_type = other DNA
cactctttccctacacgacgctcttccgatctgttttgttccagagtctatcaccg

SEQ ID NO: 41 - DNA, 52 bp, synthetic construct
  misc_feature 1..52: note = source = /note="Description of Artificial Sequence: Synthetic primer"
  source 1..52: mol_type = other DNA
ggagttcagacgtgtgctcttccgatctacacgaataagagcaaatgggaac

SEQ ID NO: 42 - DNA, 21 bp, synthetic construct
  misc_feature 1..21: note = source = /note="Description of Artificial Sequence: Synthetic primer"
  source 1..21: mol_type = other DNA
tgctgcaaggcgattaagttg

SEQ ID NO: 43 - DNA, 21 bp, synthetic construct
  misc_feature 1..21: note = source = /note="Description of Artificial Sequence: Synthetic primer"
  source 1..21: mol_type = other DNA
ttagctcactcattaggcacc

SEQ ID NO: 44 - RNA, 20 nt, synthetic construct
  misc_feature 1..20: note = source = /note="Description of Artificial Sequence: Synthetic oligonucleotide"
  source 1..20: mol_type = other RNA
tcttgtctcctctgtgccca

SEQ ID NO: 45 - RNA, 20 nt, synthetic construct
  misc_feature 1..20: note = source = /note="Description of Artificial Sequence: Synthetic oligonucleotide"
  source 1..20: mol_type = other RNA
ctcctctgtgcccagggtgc

SEQ ID NO: 46 - RNA, 20 nt, synthetic construct
  misc_feature 1..20: note = source = /note="Description of Artificial Sequence: Synthetic oligonucleotide"
  source 1..20: mol_type = other RNA
agaatccaaatgtcctctga

SEQ ID NO: 47 - RNA, 20 nt, synthetic construct
  misc_feature 1..20: note = source = /note="Description of Artificial Sequence: Synthetic oligonucleotide"
  source 1..20: mol_type = other RNA
agtgttcaaaaagacctctg

SEQ ID NO: 48 - RNA, 20 nt, synthetic construct
  misc_feature 1..20: note = source = /note="Description of Artificial Sequence: Synthetic oligonucleotide"
  source 1..20: mol_type = other RNA
aaaagacctctgagggatcc

SEQ ID NO: 49 - RNA, 20 nt, synthetic construct
  misc_feature 1..20: note = source = /note="Description of Artificial Sequence: Synthetic oligonucleotide"
  source 1..20: mol_type = other RNA
tcctgggagccctttgcctc

SEQ ID NO: 50 - RNA, 20 nt, synthetic construct
  misc_feature 1..20: note = source = /note="Description of Artificial Sequence: Synthetic oligonucleotide"
  source 1..20: mol_type = other RNA
cgtctacagcagggctgcct

SEQ ID NO: 51 - RNA, 20 nt, synthetic construct
  misc_feature 1..20: note = source = /note="Description of Artificial Sequence: Synthetic oligonucleotide"
  source 1..20: mol_type = other RNA
cccagaggcaaagggctccc

SEQ ID NO: 52 - RNA, 20 nt, synthetic construct
  misc_feature 1..20: note = source = /note="Description of Artificial Sequence: Synthetic oligonucleotide"
  source 1..20: mol_type = other RNA
ttctacaaacttctcatctg

SEQ ID NO: 53 - RNA, 20 nt, synthetic construct
  misc_feature 1..20: note = source = /note="Description of Artificial Sequence: Synthetic oligonucleotide"
  source 1..20: mol_type = other RNA
atccgcgaattcatggaacg

SEQ ID NO: 54 - RNA, 20 nt, synthetic construct
  misc_feature 1..20: note = source = /note="Description of Artificial Sequence: Synthetic oligonucleotide"
  source 1..20: mol_type = other RNA
tgtctctcctctctcctagg

SEQ ID NO: 55 - RNA, 20 nt, synthetic construct
  misc_feature 1..20: note = source = /note="Description of Artificial Sequence: Synthetic oligonucleotide"
  source 1..20: mol_type = other RNA
gttttcacagccaacgactc

SEQ ID NO: 56 - RNA, 20 nt, synthetic construct
  misc_feature 1..20: note = source = /note="Description of Artificial Sequence: Synthetic oligonucleotide"
  source 1..20: mol_type = other RNA
cccatactcctacagcacca

SEQ ID NO: 57 - RNA, 20 nt, synthetic construct
  misc_feature 1..20: note = source = /note="Description of Artificial Sequence: Synthetic oligonucleotide"
  source 1..20: mol_type = other RNA
gcagggctgcgatggtgtag

SEQ ID NO: 58 - RNA, 20 nt, synthetic construct
  misc_feature 1..20: note = source = /note="Description of Artificial Sequence: Synthetic oligonucleotide"
  source 1..20: mol_type = other RNA
tgtaggagtatgggctgagc

SEQ ID NO: 59 - RNA, 20 nt, synthetic construct
  misc_feature 1..20: note = source = /note="Description of Artificial Sequence: Synthetic oligonucleotide"
  source 1..20: mol_type = other RNA
gccgtggtgctgtaggagta

SEQ ID NO: 60 - RNA, 20 nt, synthetic construct
  misc_feature 1..20: note = source = /note="Description of Artificial Sequence: Synthetic oligonucleotide"
  source 1..20: mol_type = other RNA
tgggctgagtctctcaattc

SEQ ID NO: 61 - RNA, 20 nt, synthetic construct
  misc_feature 1..20: note = source = /note="Description of Artificial Sequence: Synthetic oligonucleotide"
  source 1..20: mol_type = other RNA
ctcttcctcctttgcctcgc

SEQ ID NO: 62 - RNA, 20 nt, synthetic construct
  misc_feature 1..20: note = source = /note="Description of Artificial Sequence: Synthetic oligonucleotide"
  source 1..20: mol_type = other RNA
ctggtatttgtgtctgaagc

SEQ ID NO: 63 - RNA, 20 nt, synthetic construct
  misc_feature 1..20: note = source = /note="Description of Artificial Sequence: Synthetic oligonucleotide"
  source 1..20: mol_type = other RNA
cctcctttgcctcgctggac

SEQ ID NO: 64 - RNA, 20 nt, synthetic construct
  misc_feature 1..20: note = source = /note="Description of Artificial Sequence: Synthetic oligonucleotide"
  source 1..20: mol_type = other RNA
ctcacaggatcactcaccgc

SEQ ID NO: 65 - RNA, 20 nt, synthetic construct
  misc_feature 1..20: note = source = /note="Description of Artificial Sequence: Synthetic oligonucleotide"
  source 1..20: mol_type = other RNA
tccacaagctcctgacagga

SEQ ID NO: 66 - RNA, 20 nt, synthetic construct
  misc_feature 1..20: note = source = /note="Description of Artificial Sequence: Synthetic oligonucleotide"
  source 1..20: mol_type = other RNA
ggcaaaggaggaagagtcga

SEQ ID NO: 67 - RNA, 20 nt, synthetic construct
  misc_feature 1..20: note = source = /note="Description of Artificial Sequence: Synthetic oligonucleotide"
  source 1..20: mol_type = other RNA
ccagtccagcgaggcaaagg

SEQ ID NO: 68 - RNA, 20 nt, synthetic construct
  misc_feature 1..20: note = source = /note="Description of Artificial Sequence: Synthetic oligonucleotide"
  source 1..20: mol_type = other RNA
ataccagtccagcgaggcaa

SEQ ID NO: 69 - RNA, 20 nt, synthetic construct
  misc_feature 1..20: note = source = /note="Description of Artificial Sequence: Synthetic oligonucleotide"
  source 1..20: mol_type = other RNA
gctcacaggatcactcaccg

SEQ ID NO: 70 - RNA, 20 nt, synthetic construct
  misc_feature 1..20: note = source = /note="Description of Artificial Sequence: Synthetic oligonucleotide"
  source 1..20: mol_type = other RNA
acacaaataccagtccagcg

SEQ ID NO: 71 - RNA, 20 nt, synthetic construct
  misc_feature 1..20: note = source = /note="Description of Artificial Sequence: Synthetic oligonucleotide"
  source 1..20: mol_type = other RNA
tcacaggatcactcaccgcg

SEQ ID NO: 72 - RNA, 20 nt, synthetic construct
  misc_feature 1..20: note = source = /note="Description of Artificial Sequence: Synthetic oligonucleotide"
  source 1..20: mol_type = other RNA
gcaaaggaggaagagtcgaa

SEQ ID NO: 73 - RNA, 20 nt, synthetic construct
  misc_feature 1..20: note = source = /note="Description of Artificial Sequence: Synthetic oligonucleotide"
  source 1..20: mol_type = other RNA
tttgaccatcagaggacatt

SEQ ID NO: 74 - RNA, 20 nt, synthetic construct
  misc_feature 1..20: note = source = /note="Description of Artificial Sequence: Synthetic oligonucleotide"
  source 1..20: mol_type = other RNA
ggctgcctcggacagcatcc

SEQ ID NO: 75 - RNA, 20 nt, synthetic construct
  misc_feature 1..20: note = source = /note="Description of Artificial Sequence: Synthetic oligonucleotide"
  source 1..20: mol_type = other RNA
tcctctgatggtcaaagtcc

SEQ ID NO: 76 - RNA, 20 nt, synthetic construct
  misc_feature 1..20: note = source = /note="Description of Artificial Sequence: Synthetic oligonucleotide"
  source 1..20: mol_type = other RNA
aaagacctctgagggatcct

SEQ ID NO: 77 - RNA, 20 nt, synthetic construct
  misc_feature 1..20: note = source = /note="Description of Artificial Sequence: Synthetic oligonucleotide"
  source 1..20: mol_type = other RNA
tttacagccacgtctacagc

SEQ ID NO: 78 - RNA, 20 nt, synthetic construct
  misc_feature 1..20: note = source = /note="Description of Artificial Sequence: Synthetic oligonucleotide"
  source 1..20: mol_type = other RNA
gtgttcaaaaagacctctga

SEQ ID NO: 79 - RNA, 20 nt, synthetic construct
  misc_feature 1..20: note = source = /note="Description of Artificial Sequence: Synthetic oligonucleotide"
  source 1..20: mol_type = other RNA
caagcttacccagaggcaaa

SEQ ID NO: 80 - RNA, 20 nt, synthetic construct
  misc_feature 1..20: note = source = /note="Description of Artificial Sequence: Synthetic oligonucleotide"
  source 1..20: mol_type = other RNA
aggcagccctgctgtagacg

SEQ ID NO: 81 - RNA, 20 nt, synthetic construct
  misc_feature 1..20: note = source = /note="Description of Artificial Sequence: Synthetic oligonucleotide"
  source 1..20: mol_type = other RNA
tccaggactttgaccatcag

SEQ ID NO: 82 - RNA, 20 nt, synthetic construct
  misc_feature 1..20: note = source = /note="Description of Artificial Sequence: Synthetic oligonucleotide"
  source 1..20: mol_type = other RNA
gggctcccaggatccctcag

SEQ ID NO: 83 - RNA, 20 nt, synthetic construct
  misc_feature 1..20: note = source = /note="Description of Artificial Sequence: Synthetic oligonucleotide"
  source 1..20: mol_type = other RNA
aaagtcctggatgctgtccg

SEQ ID NO: 84 - RNA, 20 nt, synthetic construct
  misc_feature 1..20: note = source = /note="Description of Artificial Sequence: Synthetic oligonucleotide"
  source 1..20: mol_type = other RNA
acaagcttacccagaggcaa

SEQ ID NO: 85 - RNA, 20 nt, synthetic construct
  misc_feature 1..20: note = source = /note="Description of Artificial Sequence: Synthetic oligonucleotide"
  source 1..20: mol_type = other RNA
ctttctacaagcttacccag

SEQ ID NO: 86 - RNA, 20 nt, synthetic construct
  misc_feature 1..20: note = source = /note="Description of Artificial Sequence: Synthetic oligonucleotide"
  source 1..20: mol_type = other RNA
ttacagccacgtctacagca

SEQ ID NO: 87 - RNA, 20 nt, synthetic construct
  misc_feature 1..20: note = source = /note="Description of Artificial Sequence: Synthetic oligonucleotide"
  source 1..20: mol_type = other RNA
tccaggaagaccgcggagtc

SEQ ID NO: 88 - RNA, 20 nt, synthetic construct
  misc_feature 1..20: note = source = /note="Description of Artificial Sequence: Synthetic oligonucleotide"
  source 1..20: mol_type = other RNA
cacttacatccgcgaattca

SEQ ID NO: 89 - RNA, 20 nt, synthetic construct
  misc_feature 1..20: note = source = /note="Description of Artificial Sequence: Synthetic oligonucleotide"
  source 1..20: mol_type = other RNA
aagtgtcttccagtacgatt

SEQ ID NO: 90 - RNA, 20 nt, synthetic construct
  misc_feature 1..20: note = source = /note="Description of Artificial Sequence: Synthetic oligonucleotide"
  source 1..20: mol_type = other RNA
catccgcgaattcatggaac

SEQ ID NO: 91 - RNA, 20 nt, synthetic construct
  misc_feature 1..20: note = source = /note="Description of Artificial Sequence: Synthetic oligonucleotide"
  source 1..20: mol_type = other RNA
aaatcgtactggaagacact

SEQ ID NO: 92 - RNA, 20 nt, synthetic construct
  misc_feature 1..20: note = source = /note="Description of Artificial Sequence: Synthetic oligonucleotide"
  source 1..20: mol_type = other RNA
cggagtctggagagctgcac

SEQ ID NO: 93 - RNA, 20 nt, synthetic construct
  misc_feature 1..20: note = source = /note="Description of Artificial Sequence: Synthetic oligonucleotide"
  source 1..20: mol_type = other RNA
aggagtgtacagagtagaac

SEQ ID NO: 94 - RNA, 20 nt, synthetic construct
  misc_feature 1..20: note = source = /note="Description of Artificial Sequence: Synthetic oligonucleotide"
  source 1..20: mol_type = other RNA
ttccccgttccatgaattcg

SEQ ID NO: 95 - RNA, 20 nt, synthetic construct
  misc_feature 1..20: note = source = /note="Description of Artificial Sequence: Synthetic oligonucleotide"
  source 1..20: mol_type = other RNA
acagatgagaagtttgtaga

SEQ ID NO: 96 - RNA, 20 nt, synthetic construct
  misc_feature 1..20: note = source = /note="Description of Artificial Sequence: Synthetic oligonucleotide"
  source 1..20: mol_type = other RNA
aactggacaccaaatcgtac

SEQ ID NO: 97 - RNA, 20 nt, synthetic construct
  misc_feature 1..20: note = source = /note="Description of Artificial Sequence: Synthetic oligonucleotide"
  source 1..20: mol_type = other RNA
acatccgcgaattcatggaa

SEQ ID NO: 98 - RNA, 20 nt, synthetic construct
  misc_feature 1..20: note = source = /note="Description of Artificial Sequence: Synthetic oligonucleotide"
  source 1..20: mol_type = other RNA
gcggagtctggagagctgca

SEQ ID NO: 99 - RNA, 20 nt, synthetic construct
  misc_feature 1..20: note = source = /note="Description of Artificial Sequence: Synthetic oligonucleotide"
  source 1..20: mol_type = other RNA
gtgcagctctccagactccg

SEQ ID NO: 100 - RNA, 20 nt, synthetic construct
  misc_feature 1..20: note = source = /note="Description of Artificial Sequence: Synthetic oligonucleotide"
  source 1..20: mol_type = other RNA
tgtgccctccaggaagaccg

SEQ ID NO: 101 - RNA, 20 nt, synthetic construct
  misc_feature 1..20: note = source = /note="Description of Artificial Sequence: Synthetic oligonucleotide"
  source 1..20: mol_type = other RNA
tgggctgagtctctcaattc

SEQ ID NO: 102 - RNA, 20 nt, synthetic construct
  misc_feature 1..20: note = source = /note="Description of Artificial Sequence: Synthetic oligonucleotide"
  source 1..20: mol_type = other RNA
tgtaggagtatgggctgagc

SEQ ID NO: 103 - RNA, 20 nt, synthetic construct
  misc_feature 1..20: note = source = /note="Description of Artificial Sequence: Synthetic oligonucleotide"
  source 1..20: mol_type = other RNA
tgggctgagcagggctgcga

SEQ ID NO: 104 - RNA, 20 nt, synthetic construct
  misc_feature 1..20: note = source = /note="Description of Artificial Sequence: Synthetic oligonucleotide"
  source 1..20: mol_type = other RNA
gtggcgatggccagagtcgt

SEQ ID NO: 105 - RNA, 20 nt, synthetic construct
  misc_feature 1..20: note = source = /note="Description of Artificial Sequence: Synthetic oligonucleotide"
  source 1..20: mol_type = other RNA
ctgcgatggtgtagtggcga

SEQ ID NO: 106 - RNA, 20 nt, synthetic construct
  misc_feature 1..20: note = source = /note="Description of Artificial Sequence: Synthetic oligonucleotide"
  source 1..20: mol_type = other RNA
gccgtggtgctgtaggagta

SEQ ID NO: 107 - RNA, 20 nt, synthetic construct
  misc_feature 1..20: note = source = /note="Description of Artificial Sequence: Synthetic oligonucleotide"
  source 1..20: mol_type = other RNA
ctgctcctcctctgccttgc

SEQ ID NO: 108 - RNA, 20 nt, synthetic construct
  misc_feature 1..20: note = source = /note="Description of Artificial Sequence: Synthetic oligonucleotide"
  source 1..20: mol_type = other RNA
cctcctctgccttgctggac

SEQ ID NO: 109 - RNA, 20 nt, synthetic construct
  misc_feature 1..20: note = source = /note="Description of Artificial Sequence: Synthetic oligonucleotide"
  source 1..20: mol_type = other RNA
ccagtccagcaaggcagagg

SEQ ID NO: 110 - RNA, 20 nt, synthetic construct
  misc_feature 1..20: note = source = /note="Description of Artificial Sequence: Synthetic oligonucleotide"
  source 1..20: mol_type = other RNA
ataccagtccagcaaggcag

SEQ ID NO: 111 - RNA, 20 nt, synthetic construct
  misc_feature 1..20: note = source = /note="Description of Artificial Sequence: Synthetic oligonucleotide"
  source 1..20: mol_type = other RNA
acacaaataccagtccagca

SEQ ID NO: 112 - RNA, 20 nt, synthetic construct
  misc_feature 1..20: note = source = /note="Description of Artificial Sequence: Synthetic oligonucleotide"
  source 1..20: mol_type = other RNA
tggactggtatttgtgtctg

SEQ ID NO: 113 - RNA, 20 nt, synthetic construct
  misc_feature 1..20: note = source = /note="Description of Artificial Sequence: Synthetic oligonucleotide"
  source 1..20: mol_type = other RNA
ctggtatttgtgtctgaggc

SEQ ID NO: 114 - RNA, 20 nt, synthetic construct
  misc_feature 1..20: note = source = /note="Description of Artificial Sequence: Synthetic oligonucleotide"
  source 1..20: mol_type = other RNA
cttctctacacccagggcac

SEQ ID NO: 115 - RNA, 20 nt, synthetic construct
  misc_feature 1..20: note = source = /note="Description of Artificial Sequence: Synthetic oligonucleotide"
  source 1..20: mol_type = other RNA
cagaggacacttggattcac

SEQ ID NO: 116 - RNA, 20 nt, synthetic construct
  misc_feature 1..20: note = source = /note="Description of Artificial Sequence: Synthetic oligonucleotide"
  source 1..20: mol_type = other RNA
tttgaccatcagaggacact

SEQ ID NO: 117 - RNA, 20 nt, synthetic construct
  misc_feature 1..20: note = source = /note="Description of Artificial Sequence: Synthetic oligonucleotide"
  source 1..20: mol_type = other RNA
tctagaactttgaccatcag

SEQ ID NO: 118 - RNA, 20 nt, synthetic construct
  misc_feature 1..20: note = source = /note="Description of Artificial Sequence: Synthetic oligonucleotide"
  source 1..20: mol_type = other RNA
aaagttctagatgctgtccg

SEQ ID NO: 119 - RNA, 20 nt, synthetic construct
  misc_feature 1..20: note = source = /note="Description of Artificial Sequence: Synthetic oligonucleotide"
  source 1..20: mol_type = other RNA
cattgatggcaggactgcct

SEQ ID NO: 120 - RNA, 20 nt, synthetic construct
  misc_feature 1..20: note = source = /note="Description of Artificial Sequence: Synthetic oligonucleotide"
  source 1..20: mol_type = other RNA
aggcagtcctgccatcaatg

SEQ ID NO: 121 - RNA, 20 nt, synthetic construct
  misc_feature 1..20: note = source = /note="Description of Artificial Sequence: Synthetic oligonucleotide"
  source 1..20: mol_type = other RNA
tgcacggccacattgatggc

SEQ ID NO: 122 - RNA, 20 nt, synthetic construct
  misc_feature 1..20: note = source = /note="Description of Artificial Sequence: Synthetic oligonucleotide"
  source 1..20: mol_type = other RNA
cacatgcacggccacattga

SEQ ID NO: 123 - RNA, 20 nt, synthetic construct
  misc_feature 1..20: note = source = /note="Description of Artificial Sequence: Synthetic oligonucleotide"
  source 1..20: mol_type = other RNA
agcctttctgaacacatgca

SEQ ID NO: 124 - RNA, 20 nt, synthetic construct
  misc_feature 1..20: note = source = /note="Description of Artificial Sequence: Synthetic oligonucleotide"
  source 1..20: mol_type = other RNA
gaaaggctgctgatgacacc

SEQ ID NO: 125 - RNA, 20 nt, synthetic construct
  misc_feature 1..20: note = source = /note="Description of Artificial Sequence: Synthetic oligonucleotide"
  source 1..20: mol_type = other RNA
aaaggctgctgatgacacct

SEQ ID NO: 126 - RNA, 20 nt, synthetic construct
  misc_feature 1..20: note = source = /note="Description of Artificial Sequence: Synthetic oligonucleotide"
  source 1..20: mol_type = other RNA
acctgggagccatttgcctc

SEQ ID NO: 127 - RNA, 20 nt, synthetic construct
  misc_feature 1..20: note = source = /note="Description of Artificial Sequence: Synthetic oligonucleotide"
  source 1..20: mol_type = other RNA
cccagaggcaaatggctccc

SEQ ID NO: 128 - RNA, 20 nt, synthetic construct
  misc_feature 1..20: note = source = /note="Description of Artificial Sequence: Synthetic oligonucleotide"
  source 1..20: mol_type = other RNA
gcaacttacccagaggcaaa

SEQ ID NO: 129 - RNA, 20 nt, synthetic construct
  misc_feature 1..20: note = source = /note="Description of Artificial Sequence: Synthetic oligonucleotide"
  source 1..20: mol_type = other RNA
ttctttggcaacttacccag

SEQ ID NO: 130 - RNA, 20 nt, synthetic construct
  misc_feature 1..20: note = source = /note="Description of Artificial Sequence: Synthetic oligonucleotide"
  source 1..20: mol_type = other RNA
atgcagctctccagactcac

SEQ ID NO: 131 - RNA, 20 nt, synthetic construct
  misc_feature 1..20: note = source = /note="Description of Artificial Sequence: Synthetic oligonucleotide"
  source 1..20: mol_type = other RNA
agtgagtctggagagctgca

SEQ ID NO: 132 - RNA, 20 nt, synthetic construct
  misc_feature 1..20: note = source = /note="Description of Artificial Sequence: Synthetic oligonucleotide"
  source 1..20: mol_type = other RNA
gtgagtctggagagctgcat

SEQ ID NO: 133 - RNA, 20 nt, synthetic construct
  misc_feature 1..20: note = source = /note="Description of Artificial Sequence: Synthetic oligonucleotide"
  source 1..20: mol_type = other RNA
gctgcatgggctcacaactg

SEQ ID NO: 134 - RNA, 20 nt, synthetic construct
  misc_feature 1..20: note = source = /note="Description of Artificial Sequence: Synthetic oligonucleotide"
  source 1..20: mol_type = other RNA
gcatgggctcacaactgagg

SEQ ID NO: 135 - RNA, 20 nt, synthetic construct
  misc_feature 1..20: note = source = /note="Description of Artificial Sequence: Synthetic oligonucleotide"
  source 1..20: mol_type = other RNA
actgaggaggaatttgtaga

SEQ ID NO: 136 - RNA, 20 nt, synthetic construct
  misc_feature 1..20: note = source = /note="Description of Artificial Sequence: Synthetic oligonucleotide"
  source 1..20: mol_type = other RNA
ctgaggaggaatttgtagaa

SEQ ID NO: 137 - RNA, 20 nt, synthetic construct
  misc_feature 1..20: note = source = /note="Description of Artificial Sequence: Synthetic oligonucleotide"
  source 1..20: mol_type = other RNA
tgtagaagggatatacaaag

SEQ ID NO: 138 - RNA, 20 nt, synthetic construct
  misc_feature 1..20: note = source = /note="Description of Artificial Sequence: Synthetic oligonucleotide"
  source 1..20: mol_type = other RNA
aaatagacaccaaatcttac

SEQ ID NO: 139 - RNA, 20 nt, synthetic construct
  misc_feature 1..20: note = source = /note="Description of Artificial Sequence: Synthetic oligonucleotide"
  source 1..20: mol_type = other RNA
agacaccaaatcttactgga

SEQ ID NO: 140 - RNA, 20 nt, synthetic construct
  misc_feature 1..20: note = source = /note="Description of Artificial Sequence: Synthetic oligonucleotide"
  source 1..20: mol_type = other RNA
aagtgccttccagtaagatt

SEQ ID NO: 141 - RNA, 20 nt, synthetic construct
  misc_feature 1..20: note = source = /note="Description of Artificial Sequence: Synthetic oligonucleotide"
  source 1..20: mol_type = other RNA
ctctgcatgctcatggaatg

SEQ ID NO: 142 - RNA, 20 nt, synthetic construct
  misc_feature 1..20: note = source = /note="Description of Artificial Sequence: Synthetic oligonucleotide"
  source 1..20: mol_type = other RNA
cctctgcatgctcatggaat

SEQ ID NO: 143 - RNA, 20 nt, synthetic construct
  misc_feature 1..20: note = source = /note="Description of Artificial Sequence: Synthetic oligonucleotide"
  source 1..20: mol_type = other RNA
acctctgcatgctcatggaa

SEQ ID NO: 144 - RNA, 20 nt, synthetic construct
  misc_feature 1..20: note = source = /note="Description of Artificial Sequence: Synthetic oligonucleotide"
  source 1..20: mol_type = other RNA
tactcacctctgcatgctca

SEQ ID NO: 145 - RNA, 20 nt, synthetic construct
  misc_feature 1..20: note = source = /note="Description of Artificial Sequence: Synthetic oligonucleotide"
  source 1..20: mol_type = other RNA
gtattcacagccaacgactc

SEQ ID NO: 146 - RNA, 20 nt, synthetic construct
  misc_feature 1..20: note = source = /note="Description of Artificial Sequence: Synthetic oligonucleotide"
  source 1..20: mol_type = other RNA
gcggcgggggccggagtcgt

SEQ ID NO: 147 - RNA, 20 nt, synthetic construct
  misc_feature 1..20: note = source = /note="Description of Artificial Sequence: Synthetic oligonucleotide"
  source 1..20: mol_type = other RNA
aatggtgtagcggcgggggc

SEQ ID NO: 148 - RNA, 20 nt, synthetic construct
  misc_feature 1..20: note = source = /note="Description of Artificial Sequence: Synthetic oligonucleotide"
  source 1..20: mol_type = other RNA
cggcaatggtgtagcggcgg

SEQ ID NO: 149 - RNA, 20 nt, synthetic construct
  misc_feature 1..20: note = source = /note="Description of Artificial Sequence: Synthetic oligonucleotide"
  source 1..20: mol_type = other RNA
gcggcaatggtgtagcggcg

SEQ ID NO: 150 - RNA, 20 nt, synthetic construct
  misc_feature 1..20: note = source = /note="Description of Artificial Sequence: Synthetic oligonucleotide"
  source 1..20: mol_type = other RNA
ggcggcaatggtgtagcggc

SEQ ID NO: 151 - RNA, 20 nt, synthetic construct
  misc_feature 1..20: note = source = /note="Description of Artificial Sequence: Synthetic oligonucleotide"
  source 1..20: mol_type = other RNA
gggcggcaatggtgtagcgg

SEQ ID NO: 152 - RNA, 20 nt, synthetic construct
  misc_feature 1..20: note = source = /note="Description of Artificial Sequence: Synthetic oligonucleotide"
  source 1..20: mol_type = other RNA
gcagggcggcaatggtgtag

SEQ ID NO: 153 - RNA, 20 nt, synthetic construct
  misc_feature 1..20: note = source = /note="Description of Artificial Sequence: Synthetic oligonucleotide"
  source 1..20: mol_type = other RNA
ggggctcagcagggcggcaa

SEQ ID NO: 154 - RNA, 20 nt, synthetic construct
  misc_feature 1..20: note = source = /note="Description of Artificial Sequence: Synthetic oligonucleotide"
  source 1..20: mol_type = other RNA
ggagtaggggctcagcaggg

SEQ ID NO: 155 - RNA, 20 nt, synthetic construct
  misc_feature 1..20: note = source = /note="Description of Artificial Sequence: Synthetic oligonucleotide"
  source 1..20: mol_type = other RNA
ataggagtaggggctcagca

SEQ ID NO: 156 - RNA, 20 nt, synthetic construct
  misc_feature 1..20: note = source = /note="Description of Artificial Sequence: Synthetic oligonucleotide"
  source 1..20: mol_type = other RNA
aataggagtaggggctcagc

SEQ ID NO: 157 - RNA, 20 nt, synthetic construct
  misc_feature 1..20: note = source = /note="Description of Artificial Sequence: Synthetic oligonucleotide"
  source 1..20: mol_type = other RNA
cccctactcctattccacca

SEQ ID NO: 158 - RNA, 20 nt, synthetic construct
  misc_feature 1..20: note = source = /note="Description of Artificial Sequence: Synthetic oligonucleotide"
  source 1..20: mol_type = other RNA
ccgtggtggaataggagtag

SEQ ID NO: 159 - RNA, 20 nt, synthetic construct
  misc_feature 1..20: note = source = /note="Description of Artificial Sequence: Synthetic oligonucleotide"
  source 1..20: mol_type = other RNA
gccgtggtggaataggagta

SEQ ID NO: 160 - RNA, 20 nt, synthetic construct
  misc_feature 1..20: note = source = /note="Description of Artificial Sequence: Synthetic oligonucleotide"
  source 1..20: mol_type = other RNA
gacgacagccgtggtggaat

SEQ ID NO: 161 - RNA, 20 nt, synthetic construct
  misc_feature 1..20: note = source = /note="Description of Artificial Sequence: Synthetic oligonucleotide"
  source 1..20: mol_type = other RNA
attggtgacgacagccgtgg

SEQ ID NO: 162 - RNA, 20 nt, synthetic construct
  misc_feature 1..20: note = source = /note="Description of Artificial Sequence: Synthetic oligonucleotide"
  source 1..20: mol_type = other RNA
gggattggtgacgacagccg

SEQ ID NO: 163 - RNA, 20 nt, synthetic construct
  misc_feature 1..20: note = source = /note="Description of Artificial Sequence: Synthetic oligonucleotide"
  source 1..20: mol_type = other RNA
ggctgtcgtcaccaatccca

SEQ ID NO: 164 - RNA, 20 nt, synthetic construct
  misc_feature 1..20: note = source = /note="Description of Artificial Sequence: Synthetic oligonucleotide"
  source 1..20: mol_type = other RNA
agtccctcattccttgggat